European Patent Application EP 4 585 689 A1, published July 16, 2025. Title: 신규한 유전체 세이프 하버 및 이의 용도. Applicant: 주식회사 에피바이오텍. Application KR. The sequence listing filed with the application follows.

SEQUENCE LISTING (25 sequences)

SEQ ID NO: 1 - DNA, 9174 bp, synthetic construct
  source 1..9174: mol_type = other DNA
gagggcctatttcccatgattccttcatatttgcatatacgatacaaggctgttagagagataattggaattaatttgactgtaaacacaaagatattagtacaaaatacgtgacgtagaaagtaataatttcttgggtagtttgcagttttaaaattatgttttaaaatggactatcatatgcttaccgtaacttgaaagtatttcgatttcttggctttatatatcttgtggaaaggacgaaacaccgggtcttcgagaagacctgttttagagctagaaatagcaagttaaaataaggctagtccgttatcaacttgaaaaagtggcaccgagtcggtgcttttttgttttagagctagaaatagcaagttaaaataaggctagtccgtttttagcgcgtgcgccaattctgcagacaaatggctctagaggtacccgttacataacttacggtaaatggcccgcctggctgaccgcccaacgacccccgcccattgacgtcaatagtaacgccaatagggactttccattgacgtcaatgggtggagtatttacggtaaactgcccacttggcagtacatcaagtgtatcatatgccaagtacgccccctattgacgtcaatgacggtaaatggcccgcctggcattgtgcccagtacatgaccttatgggactttcctacttggcagtacatctacgtattagtcatcgctattaccatggtcgaggtgagccccacgttctgcttcactctccccatctcccccccctccccacccccaattttgtatttatttattttttaattattttgtgcagcgatgggggcggggggggggggggggcgcgcgccaggcggggcggggcggggcgaggggcggggcggggcgaggcggagaggtgcggcggcagccaatcagagcggcgcgctccgaaagtttccttttatggcgaggcggcggcggcggcggccctataaaaagcgaagcgcgcggcgggcgggagtcgctgcgcgctgccttcgccccgtgccccgctccgccgccgcctcgcgccgcccgccccggctctgactgaccgcgttactcccacaggtgagcgggcgggacggcccttctcctccgggctgtaattagctgagcaagaggtaagggtttaagggatggttggttggtggggtattaatgtttaattacctggagcacctgcctgaaatcactttttttcaggttggaccggtgccaccatggactataaggaccacgacggagactacaaggatcatgatattgattacaaagacgatgacgataagatggccccaaagaagaagcggaaggtcggtatccacggagtcccagcagccgacaagaagtacagcatcggcctggacatcggcaccaactctgtgggctgggccgtgatcaccgacgagtacaaggtgcccagcaagaaattcaaggtgctgggcaacaccgaccggcacagcatcaagaagaacctgatcggagccctgctgttcgacagcggcgaaacagccgaggccacccggctgaagagaaccgccagaagaagatacaccagacggaagaaccggatctgctatctgcaagagatcttcagcaacgagatggccaaggtggacgacagcttcttccacagactggaagagtccttcctggtggaagaggataagaagcacgagcggcaccccatcttcggcaacatcgtggacgaggtggcctaccacgagaagtaccccaccatctaccacctgagaaagaaactggtggacagcaccgacaaggccgacctgcggctgatctatctggccctggcccacatgatcaagttccggggccacttcctgatcgagggcgacctgaaccccgacaacagcgacgtggacaagctgttcatccagctggtgcagacctacaaccagctgttcgaggaaaaccccatcaacgccagcggcgtggacgccaaggccatcctgtctgccagactgagcaagagcagacggctggaaaatctgatcgcccagctgcccggcgagaagaagaatggcctgttcggaaacctgattgccctgagcctgggcctgacccccaacttcaagagcaacttcgacctggccgaggatgccaaactgcagctgagcaaggacacctacgacgacgacctggacaacctgctggcccagatcggcgaccagtacgccgacctgtttctggccgccaagaacctgtccgacgccatcctgctgagcgacatcctgagagtgaacaccgagatcaccaaggcccccctgagcgcctctatgatcaagagatacgacgagcaccaccaggacctgaccctgctgaaagctctcgtgcggcagcagctgcctgagaagtacaaagagattttcttcgaccagagcaagaacggctacgccggctacattgacggcggagccagccaggaagagttctacaagttcatcaagcccatcctggaaaagatggacggcaccgaggaactgctcgtgaagctgaacagagaggacctgctgcggaagcagcggaccttcgacaacggcagcatcccccaccagatccacctgggagagctgcacgccattctgcggcggcaggaagatttttacccattcctgaaggacaaccgggaaaagatcgagaagatcctgaccttccgcatcccctactacgtgggccctctggccaggggaaacagcagattcgcctggatgaccagaaagagcgaggaaaccatcaccccctggaacttcgaggaagtggtggacaagggcgcttccgcccagagcttcatcgagcggatgaccaacttcgataagaacctgcccaacgagaaggtgctgcccaagcacagcctgctgtacgagtacttcaccgtgtataacgagctgaccaaagtgaaatacgtgaccgagggaatgagaaagcccgccttcctgagcggcgagcagaaaaaggccatcgtggacctgctgttcaagaccaaccggaaagtgaccgtgaagcagctgaaagaggactacttcaagaaaatcgagtgcttcgactccgtggaaatctccggcgtggaagatcggttcaacgcctccctgggcacataccacgatctgctgaaaattatcaaggacaaggacttcctggacaatgaggaaaacgaggacattctggaagatatcgtgctgaccctgacactgtttgaggacagagagatgatcgaggaacggctgaaaacctatgcccacctgttcgacgacaaagtgatgaagcagctgaagcggcggagatacaccggctggggcaggctgagccggaagctgatcaacggcatccgggacaagcagtccggcaagacaatcctggatttcctgaagtccgacggcttcgccaacagaaacttcatgcagctgatccacgacgacagcctgacctttaaagaggacatccagaaagcccaggtgtccggccagggcgatagcctgcacgagcacattgccaatctggccggcagccccgccattaagaagggcatcctgcagacagtgaaggtggtggacgagctcgtgaaagtgatgggccggcacaagcccgagaacatcgtgatcgaaatggccagagagaaccagaccacccagaagggacagaagaacagccgcgagagaatgaagcggatcgaagagggcatcaaagagctgggcagccagatcctgaaagaacaccccgtggaaaacacccagctgcagaacgagaagctgtacctgtactacctgcagaatgggcgggatatgtacgtggaccaggaactggacatcaaccggctgtccgactacgatgtggaccatatcgtgcctcagagctttctgaaggacgactccatcgacaacaaggtgctgaccagaagcgacaagaaccggggcaagagcgacaacgtgccctccgaagaggtcgtgaagaagatgaagaactactggcggcagctgctgaacgccaagctgattacccagagaaagttcgacaatctgaccaaggccgagagaggcggcctgagcgaactggataaggccggcttcatcaagagacagctggtggaaacccggcagatcacaaagcacgtggcacagatcctggactcccggatgaacactaagtacgacgagaatgacaagctgatccgggaagtgaaagtgatcaccctgaagtccaagctggtgtccgatttccggaaggatttccagttttacaaagtgcgcgagatcaacaactaccaccacgcccacgacgcctacctgaacgccgtcgtgggaaccgccctgatcaaaaagtaccctaagctggaaagcgagttcgtgtacggcgactacaaggtgtacgacgtgcggaagatgatcgccaagagcgagcaggaaatcggcaaggctaccgccaagtacttcttctacagcaacatcatgaactttttcaagaccgagattaccctggccaacggcgagatccggaagcggcctctgatcgagacaaacggcgaaaccggggagatcgtgtgggataagggccgggattttgccaccgtgcggaaagtgctgagcatgccccaagtgaatatcgtgaaaaagaccgaggtgcagacaggcggcttcagcaaagagtctatcctgcccaagaggaacagcgataagctgatcgccagaaagaaggactgggaccctaagaagtacggcggcttcgacagccccaccgtggcctattctgtgctggtggtggccaaagtggaaaagggcaagtccaagaaactgaagagtgtgaaagagctgctggggatcaccatcatggaaagaagcagcttcgagaagaatcccatcgactttctggaagccaagggctacaaagaagtgaaaaaggacctgatcatcaagctgcctaagtactccctgttcgagctggaaaacggccggaagagaatgctggcctctgccggcgaactgcagaagggaaacgaactggccctgccctccaaatatgtgaacttcctgtacctggccagccactatgagaagctgaagggctcccccgaggataatgagcagaaacagctgtttgtggaacagcacaagcactacctggacgagatcatcgagcagatcagcgagttctccaagagagtgatcctggccgacgctaatctggacaaagtgctgtccgcctacaacaagcaccgggataagcccatcagagagcaggccgagaatatcatccacctgtttaccctgaccaatctgggagcccctgccgccttcaagtactttgacaccaccatcgaccggaagaggtacaccagcaccaaagaggtgctggacgccaccctgatccaccagagcatcaccggcctgtacgagacacggatcgacctgtctcagctgggaggcgacaaaaggccggcggccacgaaaaaggccggccaggcaaaaaagaaaaaggaattcggcagtggagagggcagaggaagtctgctaacatgcggtgacgtcgaggagaatcctggcccaatgaccgagtacaagcccacggtgcgcctcgccacccgcgacgacgtccccagggccgtacgcaccctcgccgccgcgttcgccgactaccccgccacgcgccacaccgtcgatccggaccgccacatcgagcgggtcaccgagctgcaagaactcttcctcacgcgcgtcgggctcgacatcggcaaggtgtgggtcgcggacgacggcgccgcggtggcggtctggaccacgccggagagcgtcgaagcgggggcggtgttcgccgagatcggcccgcgcatggccgagttgagcggttcccggctggccgcgcagcaacagatggaaggcctcctggcgccgcaccggcccaaggagcccgcgtggttcctggccaccgtcggagtctcgcccgaccaccagggcaagggtctgggcagcgccgtcgtgctccccggagtggaggcggccgagcgcgccggggtgcccgccttcctggagacctccgcgccccgcaacctccccttctacgagcggctcggcttcaccgtcaccgccgacgtcgaggtgcccgaaggaccgcgcacctggtgcatgacccgcaagcccggtgcctgagaattctaactagagctcgctgatcagcctcgactgtgccttctagttgccagccatctgttgtttgcccctcccccgtgccttccttgaccctggaaggtgccactcccactgtcctttcctaataaaatgaggaaattgcatcgcattgtctgagtaggtgtcattctattctggggggtggggtggggcaggacagcaagggggaggattgggaagagaatagcaggcatgctggggagcggccgcaggaacccctagtgatggagttggccactccctctctgcgcgctcgctcgctcactgaggccgggcgaccaaaggtcgcccgacgcccgggctttgcccgggcggcctcagtgagcgagcgagcgcgcagctgcctgcaggggcgcctgatgcggtattttctccttacgcatctgtgcggtatttcacaccgcatacgtcaaagcaaccatagtacgcgccctgtagcggcgcattaagcgcggcgggtgtggtggttacgcgcagcgtgaccgctacacttgccagcgccttagcgcccgctcctttcgctttcttcccttcctttctcgccacgttcgccggctttccccgtcaagctctaaatcgggggctccctttagggttccgatttagtgctttacggcacctcgaccccaaaaaacttgatttgggtgatggttcacgtagtgggccatcgccctgatagacggtttttcgccctttgacgttggagtccacgttctttaatagtggactcttgttccaaactggaacaacactcaactctatctcgggctattcttttgatttataagggattttgccgatttcggtctattggttaaaaaatgagctgatttaacaaaaatttaacgcgaattttaacaaaatattaacgtttacaattttatggtgcactctcagtacaatctgctctgatgccgcatagttaagccagccccgacacccgccaacacccgctgacgcgccctgacgggcttgtctgctcccggcatccgcttacagacaagctgtgaccgtctccgggagctgcatgtgtcagaggttttcaccgtcatcaccgaaacgcgcgagacgaaagggcctcgtgatacgcctatttttataggttaatgtcatgataataatggtttcttagacgtcaggtggcacttttcggggaaatgtgcgcggaacccctatttgtttatttttctaaatacattcaaatatgtatccgctcatgagacaataaccctgataaatgcttcaataatattgaaaaaggaagagtatgagtattcaacatttccgtgtcgcccttattcccttttttgcggcattttgccttcctgtttttgctcacccagaaacgctggtgaaagtaaaagatgctgaagatcagttgggtgcacgagtgggttacatcgaactggatctcaacagcggtaagatccttgagagttttcgccccgaagaacgttttccaatgatgagcacttttaaagttctgctatgtggcgcggtattatcccgtattgacgccgggcaagagcaactcggtcgccgcatacactattctcagaatgacttggttgagtactcaccagtcacagaaaagcatcttacggatggcatgacagtaagagaattatgcagtgctgccataaccatgagtgataacactgcggccaacttacttctgacaacgatcggaggaccgaaggagctaaccgcttttttgcacaacatgggggatcatgtaactcgccttgatcgttgggaaccggagctgaatgaagccataccaaacgacgagcgtgacaccacgatgcctgtagcaatggcaacaacgttgcgcaaactattaactggcgaactacttactctagcttcccggcaacaattaatagactggatggaggcggataaagttgcaggaccacttctgcgctcggcccttccggctggctggtttattgctgataaatctggagccggtgagcgtggaagccgcggtatcattgcagcactggggccagatggtaagccctcccgtatcgtagttatctacacgacggggagtcaggcaactatggatgaacgaaatagacagatcgctgagataggtgcctcactgattaagcattggtaactgtcagaccaagtttactcatatatactttagattgatttaaaacttcatttttaatttaaaaggatctaggtgaagatcctttttgataatctcatgaccaaaatcccttaacgtgagttttcgttccactgagcgtcagaccccgtagaaaagatcaaaggatcttcttgagatcctttttttctgcgcgtaatctgctgcttgcaaacaaaaaaaccaccgctaccagcggtggtttgtttgccggatcaagagctaccaactctttttccgaaggtaactggcttcagcagagcgcagataccaaatactgttcttctagtgtagccgtagttaggccaccacttcaagaactctgtagcaccgcctacatacctcgctctgctaatcctgttaccagtggctgctgccagtggcgataagtcgtgtcttaccgggttggactcaagacgatagttaccggataaggcgcagcggtcgggctgaacggggggttcgtgcacacagcccagcttggagcgaacgacctacaccgaactgagatacctacagcgtgagctatgagaaagcgccacgcttcccgaagggagaaaggcggacaggtatccggtaagcggcagggtcggaacaggagagcgcacgagggagcttccagggggaaacgcctggtatctttatagtcctgtcgggtttcgccacctctgacttgagcgtcgatttttgtgatgctcgtcaggggggcggagcctatggaaaaacgccagcaacgcggcctttttacggttcctggccttttgctggccttttgctcacatgt

SEQ ID NO: 2 - DNA, 10760 bp, synthetic construct
  source 1..10760: mol_type = other DNA
tgcagctctggcccgtgtctcaaaatctctgatgttacattgcacaagataaaaatatatcatcatgaacaataaaactgtctgcttacataaacagtaatacaaggggtgttatgagccatattcaacgggaaacgtcgaggccgcgattaaattccaacatggatgctgatttatatgggtataaatgggctcgcgataatgtcgggcaatcaggtgcgacaatctatcgcttgtatgggaagcccgatgcgccagagttgtttctgaaacatggcaaaggtagcgttgccaatgatgttacagatgagatggtcagactaaactggctgacggaatttatgcctcttccgaccatcaagcattttatccgtactcctgatgatgcatggttactcaccactgcgatccccggaaaaacagcattccaggtattagaagaatatcctgattcaggtgaaaatattgttgatgcgctggcagtgttcctgcgccggttgcattcgattcctgtttgtaattgtccttttaacagcgatcgcgtatttcgtctcgctcaggcgcaatcacgaatgaataacggtttggttgatgcgagtgattttgatgacgagcgtaatggctggcctgttgaacaagtctggaaagaaatgcataaacttttgccattctcaccggattcagtcgtcactcatggtgatttctcacttgataaccttatttttgacgaggggaaattaataggttgtattgatgttggacgagtcggaatcgcagaccgataccaggatcttgccatcctatggaactgcctcggtgagttttctccttcattacagaaacggctttttcaaaaatatggtattgataatcctgatatgaataaattgcagtttcatttgatgctcgatgagtttttctaatcagaattggttaattggttgtaacattattcagattgggcttgatttaaaacttcatttttaatttaaaaggatctaggtgaagatcctttttgataatctcatgaccaaaatcccttaacgtgagttttcgttccactgagcgtcagaccccgtagaaaagatcaaaggatcttcttgagatcctttttttctgcgcgtaatctgctgcttgcaaacaaaaaaaccaccgctaccagcggtggtttgtttgccggatcaagagctaccaactctttttccgaaggtaactggcttcagcagagcgcagataccaaatactgttcttctagtgtagccgtagttaggccaccacttcaagaactctgtagcaccgcctacatacctcgctctgctaatcctgttaccagtggctgctgccagtggcgataagtcgtgtcttaccgggttggactcaagacgatagttaccggataaggcgcagcggtcgggctgaacggggggttcgtgcacacagcccagcttggagcgaacgacctacaccgaactgagatacctacagcgtgagctatgagaaagcgccacgcttcccgaagggagaaaggcggacaggtatccggtaagcggcagggtcggaacaggagagcgcacgagggagcttccagggggaaacgcctggtatctttatagtcctgtcgggtttcgccacctctgacttgagcgtcgatttttgtgatgctcgtcaggggggcggagcctatggaaaaacgccagcaacgcggcctttttacggttcctggccttttgctggccttttgctcacatgttctttcctgcgttatcccctgattctgtggataaccgtattaccgcctttgagtgagctgataccgctcgccgcagccgaacgaccgagcgcagcgagtcagtgagcgaggaagcggaagagcgcccaatacgcaaaccgcctctccccgcgcgttggccgattcattaatgcagctggcacgacaggtttcccgactggaaagcgggcagtgagcgcaacgcaattaatgtgagttagctcactcattaggcaccccaggctttacactttatgcttccggctcgtatgttgtgtggaattgtgagcggataacaatttcacacaggaaacagctatgaccatgattacgccgcggccgctgctttctctgaccagcattctctcccctgggcctgtgccgctttctgtctgcagcttgtggcctgggtcacctctacggctggcccagatccttccctgccgcctccttcaggttccgtcttcctccactccctcttccccttgctctctgctgtgttgctgcccaaggatgctctttccggagcacttccttctcggcgctgcaccacgtgatgtcctctgagcggatcctccccgtgtctgggtcctctccgggcatctctcctccctcacccaaccccatgccgtcttcactcgctgggttcccttttccttctccttctggggcctgtgccatctctcgtttcttaggatggccttctccgacggatgtctcccttgcgtcccgcctccccttcttgtaggcctgcatcatcaccgtttttctggacaaccccaaagtaccccgtctccctggctttagccacctctccatcctcttgctttctttgcctggacaccccgttctcctgtggattcgggtcacctctcactcctttcatttgggcagctcccctaccccccttacctctctagtctgtgctagctcttccagccccctgtcatggcatcttccaggggtccgagagctcagctagtcttcttcctccaacccgggcccctatgtccacttcaggacagcatgtttgctgcctccagggatcctgtgtccccgagctgggaccaccttatattcccagggccggttaatgtggctctggttctgggtacttttatctgtcccctccaccccacagtggggcgcggccgcataacttcgtatagcatacattatacgaagttatctgacctcttctcttcctcccacagggcctcgagagatctggcagcggagagggcagaggaagtcttctaacatgcggtgacgtggaggagaatcccggccctaggatgaccgagtacaagcccacggtgcgcctcgccacccgcgacgacgtccccagggccgtacgcaccctcgccgccgcgttcgccgactaccccgccacgcgccacaccgtcgatccggaccgccacatcgagcgggtcaccgagctgcaagaactcttcctcacgcgcgtcgggctcgacatcggcaaggtgtgggtcgcggacgacggcgccgcggtggcggtctggaccacgccggagagcgtcgaagcgggggcggtgttcgccgagatcggcccgcgcatggccgagttgagcggttcccggctggccgcgcagcaacagatggaaggcctcctggcgccgcaccggcccaaggagcccgcgtggttcctggccaccgtcggcgtctcgcccgaccaccagggcaagggtctgggcagcgccgtcgtgctccccggagtggaggcggccgagcgcgccggggtgcccgccttcctggagacctccgcgccccgcaacctccccttctacgagcggctcggcttcaccgtcaccgccgacgtcgaggtgcccgaaggaccgcgcacctggtgcatgacccgcaagcccggtgcctgactgtgccttctagttgccagccatctgttgtttgcccctcccccgtgccttccttgaccctggaaggtgccactcccactgtcctttcctaataaaatgaggaaattgcatcgcattgtctgagtaggtgtcattctattctggggggtggggtggggcaggacagcaagggggaggattgggaagacaatagcaggcatgctggggatgcggtgggctctatggataacttcgtatagcatacattatacgaagttatgagctcacggggacagcccccccccaaagcccccagggatgtaattacgtccctcccccgctagggggcagcagcgagccgcccggggctccgctccggtccggcgctccccccgcatccccgagccggcagcgtgcggggacagcccgggcacggggaaggtggcacgggatcgctttcctctgaacgcttctcgctgctctttgagcctgcagacacctggggggatacggggaaaaagctttaggctgaaagagagatttagaatgacagaatcatagaacggcctgggttgcaaaggagcacagtgctcatccagatccaaccccctgctatgtgcagggtcatcaaccagcagcccaggctgcccagagccacatccagcctggccttgaatgcctgcagggatggggcatccacagcctccttgggcaacctgttcagtgcgtcaccaccctctgggggaaaaactgcctcctcatatccaacccaaacctcccctgtctcagtgtaaagccattcccccttgtcctatcaagggggagtttgctgtgacattgttggtctggggtgacacatgtttgccaattcagtgcatcacggagaggcagatcttggggataaggaagtgcaggacagcatggacgtgggacatgcaggtgttgagggctctgggacactctccaagtcacagcgttcagaacagccttaaggataagaagataggatagaaggacaaagagcaagttaaaacccagcatggagaggagcacaaaaaggccacagacactgctggtccctgtgtctgagcctgcatgtttgatggtgtctggatgcaagcagaaggggtggaagagcttgcctggagagatacagctgggtcagtaggactgggacaggcagctggagaattgccatgtagatgttcatacaatcgtcaaatcatgaaggctggaaaagccctccaagatccccaagaccaaccccaacccacccaccgtgcccactggccatgtccctcagtgccacatccccacagttcttcatcacctccagggacggtgacccccccacctccgtgggcagctgtgccactgcagcaccgctctttggagaaggtaaatcttgctaaatccagcccgaccctcccctggcacaacgtaaggccattatctctcatccaactccaggacggagtcagtgagaatattggcgcgccgaattctcgcgacgatcggtcgacataacttcgtataggatactttatacgaagttatcaattcaggctagttattaatagtaatcaattacggggtcattagttcatagcccatatatggagttccgcgttacataacttacggtaaatggcccgcctggctgaccgcccaacgacccccgcccattgacgtcaataatgacgtatgttcccatagtaacgccaatagggactttccattgacgtcaatgggtggagtatttacggtaaactgcccacttggcagtacatcaagtgtatcatatgccaagtacgccccctattgacgtcaatgacggtaaatggcccgcctggcattatgcccagtacatgaccttatgggactttcctacttggcagtacatctacgtattagtcatcgctattaccatggtcgaggtgagccccacgttctgcttcactctccccatctcccccccctccccacccccaattttgtatttatttattttttaattattttgtgcagcgatgggggcggggggggggggggggcgcgcgccaggcggggcggggcggggcgaggggcggggcggggcgaggcggagaggtgcggcggcagccaatcagagcggcgcgctccgaaagtttccttttatggcgaggcggcggcggcggcggccctataaaaagcgaagcgcgcggcgggcggggagtcgctgcgacgctgccttcgccccgtgccccgctccgccgccgcctcgcgccgcccgccccggctctgactgaccgcgttactcccacaggtgagcgggcgggacggcccttctcctccgggctgtaattagcgcttggtttaatgacggcttgtttcttttctgtggctgcgtgaaagccttgaggggctccgggagggccctttgtgcggggggagcggctcggggggtgcgtgcgtgtgtgtgtgcgtggggagcgccgcgtgcggctccgcgctgcccggcggctgtgagcgctgcgggcgcggcgcggggctttgtgcgctccgcagtgtgcgcgaggggagcgcggccgggggcggtgccccgcggtgcggggggggctgcgaggggaacaaaggctgcgtgcggggtgtgtgcgtgggggggtgagcagggggtgtgggcgcgtcggtcgggctgcaaccccccctgcacccccctccccgagttgctgagcacggcccggcttcgggtgcggggctccgtacggggcgtggcgcggggctcgccgtgccgggcggggggtggcggcaggtgggggtgccgggcggggcggggccgcctcgggccggggagggctcgggggaggggcgcggcggcccccggagcgccggcggctgtcgaggcgcggcgagccgcagccattgccttttatggtaatcgtgcgagagggcgcagggacttcctttgtcccaaatctgtgcggagccgaaatctgggaggcgccgccgcaccccctctagcgggcgcggggcgaagcggtgcggcgccggcaggaaggaaatgggcggggagggccttcgtgcgtcgccgcgccgccgtccccttctccctctccagcctcggggctgtccgcggggggacggctgccttcgggggggacggggcagggcggggttcggcttctggcgtgtgaccggcggctctagagcctctgctaaccatgttcatgccttcttctttttcctacagctcctgggcaacgtgctggttattgtgctgtctcatcattttggcaaagaattgtgtacaaccatggagagcgacgagagcggcctgcccgccatggagatcgagtgccgcatcaccggcaccctgaacggcgtggagttcgagctggtgggcggcggagagggcacccccaagcagggccgcatgaccaacaagatgaagagcaccaaaggcgccctgaccttcagcccctacctgctgagccacgtgatgggctacggcttctaccacttcggcacctaccccagcggctacgagaaccccttcctgcacgccatcaacaacggcggctacaccaacacccgcatcgagaagtacgaggacggcggcgtgctgcacgtgagcttcagctaccgctacgaggccggccgcgtgatcggcgacttcaaggtggtgggcaccggcttccccgaggacagcgtgatcttcaccgacaagatcatccgcagcaacgccaccgtggagcacctgcaccccatgggcgataacgtgctggtgggcagcttcgcccgcaccttcagcctgcgcgacggcggctactacagcttcgtggtggacagccacatgcacttcaagagcgccatccaccccagcatcctgcagaacgggggccccatgttcgccttccgccgcgtggaggagctgcacagcaacaccgagctgggcatcgtggagtaccagcacgccttcaagacccccatcgccttcgccagatcccgcgctcagtcgtccaattctgccgtggacggcaccgccggacccggctccaccggatctcgctaaacgcgtgaattcactcctcaggtgcaggctgcctatcagaaggtggtggctggtgtggccaatgccctggctcacaaataccactgagatctttttccctctgccaaaaattatggggacatcatgaagccccttgagcatctgacttctggctaataaaggaaatttattttcattgcaatagtgtgttggaattttttgtgtctctcactcggaaggacatatgggagggcaaatcatttaaaacatcagaatgagtatttggtttagagtttggcaacatatgcccatatgctggctgccatgaacaaaggttggctataaagaggtcatcagtatatgaaacagccccctgctgtccattccttattccatagaaaagccttgacttgaggttagattttttttatattttgttttgtgttatttttttctttaacatccctaaaattttccttacatgttttactagccagatttttcctcctctcctgactactcccagtcatagctgtccctcttctcttatggagatcaccggtataacttcgtataatgtatactatacgaagttatggtaccttaattaagttaacatgcatagtactgagctcacggggacagcccccccccaaagcccccagggatgtaattacgtccctcccccgctagggggcagcagcgagccgcccggggctccgctccggtccggcgctccccccgcatccccgagccggcagcgtgcggggacagcccgggcacggggaaggtggcacgggatcgctttcctctgaacgcttctcgctgctctttgagcctgcagacacctggggggatacggggaaaaagctttaggctgaaagagagatttagaatgacagaatcatagaacggcctgggttgcaaaggagcacagtgctcatccagatccaaccccctgctatgtgcagggtcatcaaccagcagcccaggctgcccagagccacatccagcctggccttgaatgcctgcagggatggggcatccacagcctccttgggcaacctgttcagtgcgtcaccaccctctgggggaaaaactgcctcctcatatccaacccaaacctcccctgtctcagtgtaaagccattcccccttgtcctatcaagggggagtttgctgtgacattgttggtctggggtgacacatgtttgccaattcagtgcatcacggagaggcagatcttggggataaggaagtgcaggacagcatggacgtgggacatgcaggtgttgagggctctgggacactctccaagtcacagcgttcagaacagccttaaggataagaagataggatagaaggacaaagagcaagttaaaacccagcatggagaggagcacaaaaaggccacagacactgctggtccctgtgtctgagcctgcatgtttgatggtgtctggatgcaagcagaaggggtggaagagcttgcctggagagatacagctgggtcagtaggactgggacaggcagctggagaattgccatgtagatgttcatacaatcgtcaaatcatgaaggctggaaaagccctccaagatccccaagaccaaccccaacccacccaccgtgcccactggccatgtccctcagtgccacatccccacagttcttcatcacctccagggacggtgacccccccacctccgtgggcagctgtgccactgcagcaccgctctttggagaaggtaaatcttgctaaatccagcccgaccctcccctggcacaacgtaaggccattatctctcatccaactccaggacggagtcagtgagaatattgtttaaacactagggacaggattggtgacagaaaagccccatccttaggcctcctccttcctagtctcctgatattgggtctaacccccacctcctgttaggcagattccttatctggtgacacacccccatttcctggagccatctctctccttgccagaacctctaaggtttgcttacgatggagccagagaggatcctgggagggagagcttggcagggggtgggagggaagggggggatgcgtgacctgcccggttctcagtggccaccctgcgctaccctctcccagaacctgagctgctctgacgcggctgtctggtgcgtttcactgatcctggtgctgcagcttccttacacttcccaagaggagaagcagtttggaaaaacaaaatcagaataagttggtcctgagttctaactttggctcttcacctttctagtccccaatttatattgttcctccgtgcgtcagttttacctgtgagataaggccagtagccagccccgtcctggcagggctgtggtgaggaggggggtgtccgtgtggaaaactccctttgtgagaatggtgcgtcctaggtgttcaccaggtcgtggccgcctctactccctttctctttctccatccttctttccttaaagagtccccagtgctatctgggacatattcctccgcccagagcagggtcccgcttccctaaggccctgctctgggcttctgggtttgagtccttggcaagcccaggagaggcgctcaggcttccctgtcccccttcctcgtccaccatctcatgcccctggctctcctgccccttccctacaggggttcctggctctgctctgtttaaacactggccgtcgttttacaacgtcgtgactgggaaaaccctggcgttacccaacttaatcgccttgcagcacatccccctttcgccagctggcgtaatagcgaagaggcccgcaccgatcgcccttcccaacagttgcgcagcctgaatggcgaatggcgcctgatgcggtattttctccttacgcatctgtgcggtatttcacaccgcatatggtgcactctcagtacaatctgctctgatgccgcatagttaagccagccccgacacccgccaacacccgctgacgcgccctgacgggcttgtctgctcccggcatccgcttacagacaagctgtgaccgtctccgggagctgcatgtgtcagaggttttcaccgtcatcaccgaaacgcgcga

SEQ ID NO: 3 - DNA, 20 bp, synthetic construct
  source 1..20: mol_type = other DNA
cttcagtgctctactcttgt

SEQ ID NO: 4 - DNA, 20 bp, synthetic construct
  source 1..20: mol_type = other DNA
gtaagcaaaccacaacgtct

SEQ ID NO: 5 - DNA, 20 bp, synthetic construct
  source 1..20: mol_type = other DNA
tctgagacagctaatatcat

SEQ ID NO: 6 - DNA, 24 bp, synthetic construct
  source 1..24: mol_type = other DNA
caccgttcagtgctctactcttgt

SEQ ID NO: 7 - DNA, 24 bp, synthetic construct
  source 1..24: mol_type = other DNA
aaacacaagagtagagcactgaac

SEQ ID NO: 8 - DNA, 24 bp, synthetic construct
  source 1..24: mol_type = other DNA
caccgtaagcaaaccacaacgtct

SEQ ID NO: 9 - DNA, 24 bp, synthetic construct
  source 1..24: mol_type = other DNA
aaacagacgttgtggtttgcttac

SEQ ID NO: 10 - DNA, 24 bp, synthetic construct
  source 1..24: mol_type = other DNA
caccgtctgagacagctaatatca

SEQ ID NO: 11 - DNA, 24 bp, synthetic construct
  source 1..24: mol_type = other DNA
aaactgatattagctgtctcagac

SEQ ID NO: 12 - DNA, 23 bp, synthetic construct
  source 1..23: mol_type = other DNA
accgtcccctccaccccacagtg

SEQ ID NO: 13 - DNA, 23 bp, synthetic construct
  source 1..23: mol_type = other DNA
aaccactgtggggtggaggggac

SEQ ID NO: 14 - DNA, 806 bp, synthetic construct
  source 1..806: mol_type = other DNA
tgtgggaagcttctttccaacttggttcctgtccatacccacgtaaaatattaaagaaagaaggatagaaatatagattaaaagaagacctgaagtcgaaggaagggactaattgttgagagatttgaaatgcaaccaattttccatcagatgttttatcggtactctgtagttctattccgtcccagttttccataaatttatagataaaaagaatattttatattgcattttgtatgcatatatgcatacatacatatcacttaaatatatatatatataaaattgcatgttatgcacactttaaaatctttaaaatattgaatgcttaattacttaggacaaaatagcttacataggaaacaattatttcggacagaataatttaggagacaatagcatttttgtgctgttgcagagatgataaagaacttctggttttatatgtaactctaaaactgcaggataaataggtacgtaatacaaatggcagttgcctcactgcaattttctgagctgtgttgctagtctgacactcctgaaaattaatatttcagacatctctgtaattgtccagagggcctggagtgccttcaaattatattccccctctattttaatcaaccatgttagtaatttacttttcattagtttattgataattctatagggaaagtttgctaatcactgtgtaaaatataattttcaaacagccaaaataactgccataaaatatggaaactgtcttagtttgttttctcttgctatgaaagaataccacagactgggtaatgtatagagaagag

SEQ ID NO: 15 - DNA, 828 bp, synthetic construct
  source 1..828: mol_type = other DNA
gcaaatagcaagtcttctctggttctttgagctctgtttttgatgacttcaccctggaggtaacagctttcctaaggcctgacatgcaggcctgctgcattgcaaactccctctgctcatttttggcaggttgtgctgatttatggggctatttgatttatttaatgtaccatgcctttgattgcatatactctatagcagtcactcaaaatgcaaacaaacacatcatatgttctttaattactcccatcccccttattatcaatcactgccaatatcagcagaatggctgtgattcatgctataaaattaaggtcagcaaacttgggttttgcagaagtgaatagcagcaattctgtttatattctttaatgtttcaattctaaaactcattatcagaaaaatggtatttcagatcagtcttgttagaagaatgggatgggaaaaaagatataacagttgggcaaagagaaggaaagcaaatgtagcactagggaaaaagttgtagaagaaagtaaaaaaaaaaataaagatgagaagatagtagctcttaaggatattcattctgacttatgaaagactgtaatgtttagcacacacagacacatacacaaacacatgaacttgtaaaattctcaaaggtccagtttttattcaaaattcctatacttcaacttcttgaatctcactcctttttttttcaagttcctcatttctctcccttaaaaaatggatgctaaccattttaagcttagtaattttgtacatgcttttctggaaatactacaaatatgatcaatgtctgtgatctcttcagtgctctactct

SEQ ID NO: 16 - DNA, 837 bp, synthetic construct
  source 1..837: mol_type = other DNA
tctaggccaaatctggcctcccaattgttttataaataaaattttatttaaacgtaaccactcccattcatttgcttgtctctggttgtttttgcaatacaacagtagggttaggtagataatacaggctgtgtgtcacatgatgaagccaaaaacatttgctctctggctctttacagaatgaatttgcttatatttcttctaggatgtcaatttgtctgcttaattcacagaaggacaaattttaacataacttacttctatggcctgaatgtttgcgtacactgaaaattgatttgttgaaatcgatccccaatttgatagtattaggaggtagggctttggagatgtgattagatcatgagggtgtaacctttattaatgggattagtgcttttatatggggttgaagagacccgagctccccttccaccttgtgaggatgcagaaagaagatacattctgtgaactggaaagccggccctcactagacaccaaatatgccagtattttgatcttgggcttcccagccttcagaacttacagcagtccagaaagattaagacacccacctgaaatgttaattttgtcctaaaataatcttgcatttaagatctgaaatatgacctaagtattatctgaggagtcaatgctgatttattggtggtggatactgtgattctgtattaagaatggatctgaagccacataagataactgtgattacttagtgctattttcaatggctgtgagaagacaaccttgtgaccagaatttgaaaccctgcataaacaaaactcaacatgttttgaaggcctttacactcttcctctcagg

SEQ ID NO: 17 - DNA, 805 bp, synthetic construct
  source 1..805: mol_type = other DNA
cagacacatgttccccagaagaggatttgccattctgacaaatctccatccaaggaatgggaaattcattatcccttccactagaattaaactgtgaaattatttatgtaggaagaagtagtagtagaaaagttatgtttgtcttcttcactataagaaaaaaatgcaaaatcaggaaaaatgtatctaaactattacttttacaaaggcaaaaacagcctgtttgctatctaatcagtcctgttgataaaactcaggctgtactgttctcttcagagagaggcaaatggggggagttataagatttgcgccctactgctgttagtagaatgaacaagacagagtaaaagccacaagtggaattgtgctagtatttcctctataattaacccaacacttaggtagcctttaaagtgaaaggagccctccaaatgatggaggcacacaggaggtaattatgtgctttcaataaatgcctgaaagctcacaatttctttggggagatacaatctctggaaaggcttgcattgtcactccaatttcatttatttattttaacaaattgtatgttctgtggaggaactttatttcccaaaaagatgaacgtataataaaccagttctttattttaaaacttatggtgagagaaatttcaattttagataattccattgtctataaagagtctctattaaattagcttaagttccaaaagataatgccacattattattgtaggtagccattataattctcaaatttctattgttacattctgcaagacagtggtaagcaaaccacaacg

SEQ ID NO: 18 - DNA, 828 bp, synthetic construct
  source 1..828: mol_type = other DNA
tcatgggccaaaatgaatggaatcaaaacctgagacacatttctgttaatggggctctatttgagaaatgtgcattattttatcagcttccttattttaaccattctaccctgtcaatactaataccaagtgttcattttctttattagtttaaatgggagaaaacaatgcagaaagcttaataactgttctatttttaaagcctttatagaaaacataatataaaaagtgatatgaactaggcacaagacaaaactgactttaatatgttatatgttaatctgttaaaatacagtacattttactgcagaatgttagcagggtatatttgtagataatagatcattgacatttttatcctatatcctttttaccttttattccttttaaacattgattacctttgttataaaaagcaacaacaatagtttgtaaaagattaagatatttaaatatttaaaaatttttcataactatattagtaaacagtagtacataagtcttgataggtacaaatgatgtctcaaaagacagatgaggtggaaaattaccactctagctcatggcatgaccccagccgtgcagaggaaagatttcttctcctcccctattcacctccgggtcccagctatcactaaatatatcgggggtcgcgttgctgatcagcagccttaagcctgaacatggtgggtcctttgcattagttctcaattcccaccaccctcctcccttcctgtgtcacgaggctcactcatttcctcagtgcccttcccagttactgtcaaatcatataaactcatttctctgcctccagccttttatttcatc

SEQ ID NO: 19 - DNA, 860 bp, synthetic construct
  source 1..860: mol_type = other DNA
ggcttccctctgtgatgggtagataattttgcttaatatgtaaacagtcttttcaacactctgtgcttaaataatcattgttggtttgctttcttctagtattccatattaagtaatgacttggctaatgagaaggatgcttgtaagtatattagcatcaagttcaaatatagagagattaaataaccttcccaaggtcaacacactggtcattgacaaatatggaccagatctcatctccaaaaccccacacaattataccaggttagctcattctttcttcctagacatcttattttccagggagtagtgaaggtctacaaaactttcctactaaataggaaatatattttgttgtcagatgtaagcccagaaaagcaatggctaaactgctatgtatcaaaaactttgcaaacttataacagtttaaaatttacttctagctatgtttagagccctaaggagataatggcaagtcattttttcttctttatacatatgtcatcatttatggacagaaaatagttctcaattgtaaaaaaatagctctctataggatttgctgagttttttatggctagagttattaagtaaaataaatgacatctgagagcactctgctttgtctttggcttcaaataatgtattttactatattttttcattcttcgctgccataagtggcagaaagaaaaccgcttttcaaatggctagtgcctaaaaagcaaatactttgtggatcttggggccagtgtaaactcagaatgcaagatatcttcctcagcttcagtacttgcacaatgcctgtctttattaaacatgagtgatttgcaaatatgatgtttctgagacagctaata

SEQ ID NO: 20 - DNA, 837 bp, synthetic construct
  source 1..837: mol_type = other DNA
actagggacaggattggtgacagaaaagccccatccttaggcctcctccttcctagtctcctgatattgggtctaacccccacctcctgttaggcagattccttatctggtgacacacccccatttcctggagccatctctctccttgccagaacctctaaggtttgcttacgatggagccagagaggatcctgggagggagagcttggcagggggtgggagggaagggggggatgcgtgacctgcccggttctcagtggccaccctgcgctaccctctcccagaacctgagctgctctgacgcggctgtctggtgcgtttcactgatcctggtgctgcagcttccttacacttcccaagaggagaagcagtttggaaaaacaaaatcagaataagttggtcctgagttctaactttggctcttcacctttctagtccccaatttatattgttcctccgtgcgtcagttttacctgtgagataaggccagtagccagccccgtcctggcagggctgtggtgaggaggggggtgtccgtgtggaaaactccctttgtgagaatggtgcgtcctaggtgttcaccaggtcgtggccgcctctactccctttctctttctccatccttctttccttaaagagtccccagtgctatctgggacatattcctccgcccagagcagggtcccgcttccctaaggccctgctctgggcttctgggtttgagtccttggcaagcccaggagaggcgctcaggcttccctgtcccccttcctcgtccaccatctcatgcccctggctctcctgccccttccctacaggggttcctggctctgctct

SEQ ID NO: 21 - DNA, 804 bp, synthetic construct
  source 1..804: mol_type = other DNA
tgctttctctgaccagcattctctcccctgggcctgtgccgctttctgtctgcagcttgtggcctgggtcacctctacggctggcccagatccttccctgccgcctccttcaggttccgtcttcctccactccctcttccccttgctctctgctgtgttgctgcccaaggatgctctttccggagcacttccttctcggcgctgcaccacgtgatgtcctctgagcggatcctccccgtgtctgggtcctctccgggcatctctcctccctcacccaaccccatgccgtcttcactcgctgggttcccttttccttctccttctggggcctgtgccatctctcgtttcttaggatggccttctccgacggatgtctcccttgcgtcccgcctccccttcttgtaggcctgcatcatcaccgtttttctggacaaccccaaagtaccccgtctccctggctttagccacctctccatcctcttgctttctttgcctggacaccccgttctcctgtggattcgggtcacctctcactcctttcatttgggcagctcccctaccccccttacctctctagtctgtgctagctcttccagccccctgtcatggcatcttccaggggtccgagagctcagctagtcttcttcctccaacccgggcccctatgtccacttcaggacagcatgtttgctgcctccagggatcctgtgtccccgagctgggaccaccttatattcccagggccggttaatgtggctctggttctgggtacttttatctgtcccctccaccccacagtggggc

SEQ ID NO: 22 - DNA, 10753 bp, synthetic construct
  source 1..10753: mol_type = other DNA
tgcagctctggcccgtgtctcaaaatctctgatgttacattgcacaagataaaaatatatcatcatgaacaataaaactgtctgcttacataaacagtaatacaaggggtgttatgagccatattcaacgggaaacgtcgaggccgcgattaaattccaacatggatgctgatttatatgggtataaatgggctcgcgataatgtcgggcaatcaggtgcgacaatctatcgcttgtatgggaagcccgatgcgccagagttgtttctgaaacatggcaaaggtagcgttgccaatgatgttacagatgagatggtcagactaaactggctgacggaatttatgcctcttccgaccatcaagcattttatccgtactcctgatgatgcatggttactcaccactgcgatccccggaaaaacagcattccaggtattagaagaatatcctgattcaggtgaaaatattgttgatgcgctggcagtgttcctgcgccggttgcattcgattcctgtttgtaattgtccttttaacagcgatcgcgtatttcgtctcgctcaggcgcaatcacgaatgaataacggtttggttgatgcgagtgattttgatgacgagcgtaatggctggcctgttgaacaagtctggaaagaaatgcataaacttttgccattctcaccggattcagtcgtcactcatggtgatttctcacttgataaccttatttttgacgaggggaaattaataggttgtattgatgttggacgagtcggaatcgcagaccgataccaggatcttgccatcctatggaactgcctcggtgagttttctccttcattacagaaacggctttttcaaaaatatggtattgataatcctgatatgaataaattgcagtttcatttgatgctcgatgagtttttctaatcagaattggttaattggttgtaacattattcagattgggcttgatttaaaacttcatttttaatttaaaaggatctaggtgaagatcctttttgataatctcatgaccaaaatcccttaacgtgagttttcgttccactgagcgtcagaccccgtagaaaagatcaaaggatcttcttgagatcctttttttctgcgcgtaatctgctgcttgcaaacaaaaaaaccaccgctaccagcggtggtttgtttgccggatcaagagctaccaactctttttccgaaggtaactggcttcagcagagcgcagataccaaatactgttcttctagtgtagccgtagttaggccaccacttcaagaactctgtagcaccgcctacatacctcgctctgctaatcctgttaccagtggctgctgccagtggcgataagtcgtgtcttaccgggttggactcaagacgatagttaccggataaggcgcagcggtcgggctgaacggggggttcgtgcacacagcccagcttggagcgaacgacctacaccgaactgagatacctacagcgtgagctatgagaaagcgccacgcttcccgaagggagaaaggcggacaggtatccggtaagcggcagggtcggaacaggagagcgcacgagggagcttccagggggaaacgcctggtatctttatagtcctgtcgggtttcgccacctctgacttgagcgtcgatttttgtgatgctcgtcaggggggcggagcctatggaaaaacgccagcaacgcggcctttttacggttcctggccttttgctggccttttgctcacatgttctttcctgcgttatcccctgattctgtggataaccgtattaccgcctttgagtgagctgataccgctcgccgcagccgaacgaccgagcgcagcgagtcagtgagcgaggaagcggaagagcgcccaatacgcaaaccgcctctccccgcgcgttggccgattcattaatgcagctggcacgacaggtttcccgactggaaagcgggcagtgagcgcaacgcaattaatgtgagttagctcactcattaggcaccccaggctttacactttatgcttccggctcgtatgttgtgtggaattgtgagcggataacaatttcacacaggaaacagctatgaccatgattacgccgcggccgcgcaaatagcaagtcttctctggttctttgagctctgtttttgatgacttcaccctggaggtaacagctttcctaaggcctgacatgcaggcctgctgcattgcaaactccctctgctcatttttggcaggttgtgctgatttatggggctatttgatttatttaatgtaccatgcctttgattgcatatactctatagcagtcactcaaaatgcaaacaaacacatcatatgttctttaattactcccatcccccttattatcaatcactgccaatatcagcagaatggctgtgattcatgctataaaattaaggtcagcaaacttgggttttgcagaagtgaatagcagcaattctgtttatattctttaatgtttcaattctaaaactcattatcagaaaaatggtatttcagatcagtcttgttagaagaatgggatgggaaaaaagatataacagttgggcaaagagaaggaaagcaaatgtagcactagggaaaaagttgtagaagaaagtaaaaaaaaaaataaagatgagaagatagtagctcttaaggatattcattctgacttatgaaagactgtaatgtttagcacacacagacacatacacaaacacatgaacttgtaaaattctcaaaggtccagtttttattcaaaattcctatacttcaacttcttgaatctcactcctttttttttcaagttcctcatttctctcccttaaaaaatggatgctaaccattttaagcttagtaattttgtacatgcttttctggaaatactacaaatatgatcaatgtctgtgatctcttcagtgctctactctgcggccgcataacttcgtatagcatacattatacgaagttatctgacctcttctcttcctcccacagggcctcgagagatctggcagcggagagggcagaggaagtcttctaacatgcggtgacgtggaggagaatcccggccctaggatgaccgagtacaagcccacggtgcgcctcgccacccgcgacgacgtccccagggccgtacgcaccctcgccgccgcgttcgccgactaccccgccacgcgccacaccgtcgatccggaccgccacatcgagcgggtcaccgagctgcaagaactcttcctcacgcgcgtcgggctcgacatcggcaaggtgtgggtcgcggacgacggcgccgcggtggcggtctggaccacgccggagagcgtcgaagcgggggcggtgttcgccgagatcggcccgcgcatggccgagttgagcggttcccggctggccgcgcagcaacagatggaaggcctcctggcgccgcaccggcccaaggagcccgcgtggttcctggccaccgtcggcgtctcgcccgaccaccagggcaagggtctgggcagcgccgtcgtgctccccggagtggaggcggccgagcgcgccggggtgcccgccttcctggagacctccgcgccccgcaacctccccttctacgagcggctcggcttcaccgtcaccgccgacgtcgaggtgcccgaaggaccgcgcacctggtgcatgacccgcaagcccggtgcctgactgtgccttctagttgccagccatctgttgtttgcccctcccccgtgccttccttgaccctggaaggtgccactcccactgtcctttcctaataaaatgaggaaattgcatcgcattgtctgagtaggtgtcattctattctggggggtggggtggggcaggacagcaagggggaggattgggaagacaatagcaggcatgctggggatgcggtgggctctatggataacttcgtatagcatacattatacgaagttatgagctcacggggacagcccccccccaaagcccccagggatgtaattacgtccctcccccgctagggggcagcagcgagccgcccggggctccgctccggtccggcgctccccccgcatccccgagccggcagcgtgcggggacagcccgggcacggggaaggtggcacgggatcgctttcctctgaacgcttctcgctgctctttgagcctgcagacacctggggggatacggggaaaaagctttaggctgaaagagagatttagaatgacagaatcatagaacggcctgggttgcaaaggagcacagtgctcatccagatccaaccccctgctatgtgcagggtcatcaaccagcagcccaggctgcccagagccacatccagcctggccttgaatgcctgcagggatggggcatccacagcctccttgggcaacctgttcagtgcgtcaccaccctctgggggaaaaactgcctcctcatatccaacccaaacctcccctgtctcagtgtaaagccattcccccttgtcctatcaagggggagtttgctgtgacattgttggtctggggtgacacatgtttgccaattcagtgcatcacggagaggcagatcttggggataaggaagtgcaggacagcatggacgtgggacatgcaggtgttgagggctctgggacactctccaagtcacagcgttcagaacagccttaaggataagaagataggatagaaggacaaagagcaagttaaaacccagcatggagaggagcacaaaaaggccacagacactgctggtccctgtgtctgagcctgcatgtttgatggtgtctggatgcaagcagaaggggtggaagagcttgcctggagagatacagctgggtcagtaggactgggacaggcagctggagaattgccatgtagatgttcatacaatcgtcaaatcatgaaggctggaaaagccctccaagatccccaagaccaaccccaacccacccaccgtgcccactggccatgtccctcagtgccacatccccacagttcttcatcacctccagggacggtgacccccccacctccgtgggcagctgtgccactgcagcaccgctctttggagaaggtaaatcttgctaaatccagcccgaccctcccctggcacaacgtaaggccattatctctcatccaactccaggacggagtcagtgagaatattggcgcgccgaattctcgcgacgatcggtcgacataacttcgtataggatactttatacgaagttatcaattcaggctagttattaatagtaatcaattacggggtcattagttcatagcccatatatggagttccgcgttacataacttacggtaaatggcccgcctggctgaccgcccaacgacccccgcccattgacgtcaataatgacgtatgttcccatagtaacgccaatagggactttccattgacgtcaatgggtggagtatttacggtaaactgcccacttggcagtacatcaagtgtatcatatgccaagtacgccccctattgacgtcaatgacggtaaatggcccgcctggcattatgcccagtacatgaccttatgggactttcctacttggcagtacatctacgtattagtcatcgctattaccatggtcgaggtgagccccacgttctgcttcactctccccatctcccccccctccccacccccaattttgtatttatttattttttaattattttgtgcagcgatgggggcggggggggggggggggcgcgcgccaggcggggcggggcggggcgaggggcggggcggggcgaggcggagaggtgcggcggcagccaatcagagcggcgcgctccgaaagtttccttttatggcgaggcggcggcggcggcggccctataaaaagcgaagcgcgcggcgggcggggagtcgctgcgacgctgccttcgccccgtgccccgctccgccgccgcctcgcgccgcccgccccggctctgactgaccgcgttactcccacaggtgagcgggcgggacggcccttctcctccgggctgtaattagcgcttggtttaatgacggcttgtttcttttctgtggctgcgtgaaagccttgaggggctccgggagggccctttgtgcggggggagcggctcggggggtgcgtgcgtgtgtgtgtgcgtggggagcgccgcgtgcggctccgcgctgcccggcggctgtgagcgctgcgggcgcggcgcggggctttgtgcgctccgcagtgtgcgcgaggggagcgcggccgggggcggtgccccgcggtgcggggggggctgcgaggggaacaaaggctgcgtgcggggtgtgtgcgtgggggggtgagcagggggtgtgggcgcgtcggtcgggctgcaaccccccctgcacccccctccccgagttgctgagcacggcccggcttcgggtgcggggctccgtacggggcgtggcgcggggctcgccgtgccgggcggggggtggcggcaggtgggggtgccgggcggggcggggccgcctcgggccggggagggctcgggggaggggcgcggcggcccccggagcgccggcggctgtcgaggcgcggcgagccgcagccattgccttttatggtaatcgtgcgagagggcgcagggacttcctttgtcccaaatctgtgcggagccgaaatctgggaggcgccgccgcaccccctctagcgggcgcggggcgaagcggtgcggcgccggcaggaaggaaatgggcggggagggccttcgtgcgtcgccgcgccgccgtccccttctccctctccagcctcggggctgtccgcggggggacggctgccttcgggggggacggggcagggcggggttcggcttctggcgtgtgaccggcggctctagagcctctgctaaccatgttcatgccttcttctttttcctacagctcctgggcaacgtgctggttattgtgctgtctcatcattttggcaaagaattgtgtacaaccatggagagcgacgagagcggcctgcccgccatggagatcgagtgccgcatcaccggcaccctgaacggcgtggagttcgagctggtgggcggcggagagggcacccccaagcagggccgcatgaccaacaagatgaagagcaccaaaggcgccctgaccttcagcccctacctgctgagccacgtgatgggctacggcttctaccacttcggcacctaccccagcggctacgagaaccccttcctgcacgccatcaacaacggcggctacaccaacacccgcatcgagaagtacgaggacggcggcgtgctgcacgtgagcttcagctaccgctacgaggccggccgcgtgatcggcgacttcaaggtggtgggcaccggcttccccgaggacagcgtgatcttcaccgacaagatcatccgcagcaacgccaccgtggagcacctgcaccccatgggcgataacgtgctggtgggcagcttcgcccgcaccttcagcctgcgcgacggcggctactacagcttcgtggtggacagccacatgcacttcaagagcgccatccaccccagcatcctgcagaacgggggccccatgttcgccttccgccgcgtggaggagctgcacagcaacaccgagctgggcatcgtggagtaccagcacgccttcaagacccccatcgccttcgccagatcccgcgctcagtcgtccaattctgccgtggacggcaccgccggacccggctccaccggatctcgctaaacgcgtgaattcactcctcaggtgcaggctgcctatcagaaggtggtggctggtgtggccaatgccctggctcacaaataccactgagatctttttccctctgccaaaaattatggggacatcatgaagccccttgagcatctgacttctggctaataaaggaaatttattttcattgcaatagtgtgttggaattttttgtgtctctcactcggaaggacatatgggagggcaaatcatttaaaacatcagaatgagtatttggtttagagtttggcaacatatgcccatatgctggctgccatgaacaaaggttggctataaagaggtcatcagtatatgaaacagccccctgctgtccattccttattccatagaaaagccttgacttgaggttagattttttttatattttgttttgtgttatttttttctttaacatccctaaaattttccttacatgttttactagccagatttttcctcctctcctgactactcccagtcatagctgtccctcttctcttatggagatcaccggtataacttcgtataatgtatactatacgaagttatggtaccttaattaagttaacatgcatagtactgagctcacggggacagcccccccccaaagcccccagggatgtaattacgtccctcccccgctagggggcagcagcgagccgcccggggctccgctccggtccggcgctccccccgcatccccgagccggcagcgtgcggggacagcccgggcacggggaaggtggcacgggatcgctttcctctgaacgcttctcgctgctctttgagcctgcagacacctggggggatacggggaaaaagctttaggctgaaagagagatttagaatgacagaatcatagaacggcctgggttgcaaaggagcacagtgctcatccagatccaaccccctgctatgtgcagggtcatcaaccagcagcccaggctgcccagagccacatccagcctggccttgaatgcctgcagggatggggcatccacagcctccttgggcaacctgttcagtgcgtcaccaccctctgggggaaaaactgcctcctcatatccaacccaaacctcccctgtctcagtgtaaagccattcccccttgtcctatcaagggggagtttgctgtgacattgttggtctggggtgacacatgtttgccaattcagtgcatcacggagaggcagatcttggggataaggaagtgcaggacagcatggacgtgggacatgcaggtgttgagggctctgggacactctccaagtcacagcgttcagaacagccttaaggataagaagataggatagaaggacaaagagcaagttaaaacccagcatggagaggagcacaaaaaggccacagacactgctggtccctgtgtctgagcctgcatgtttgatggtgtctggatgcaagcagaaggggtggaagagcttgcctggagagatacagctgggtcagtaggactgggacaggcagctggagaattgccatgtagatgttcatacaatcgtcaaatcatgaaggctggaaaagccctccaagatccccaagaccaaccccaacccacccaccgtgcccactggccatgtccctcagtgccacatccccacagttcttcatcacctccagggacggtgacccccccacctccgtgggcagctgtgccactgcagcaccgctctttggagaaggtaaatcttgctaaatccagcccgaccctcccctggcacaacgtaaggccattatctctcatccaactccaggacggagtcagtgagaatattgtttaaactgtgggaagcttctttccaacttggttcctgtccatacccacgtaaaatattaaagaaagaaggatagaaatatagattaaaagaagacctgaagtcgaaggaagggactaattgttgagagatttgaaatgcaaccaattttccatcagatgttttatcggtactctgtagttctattccgtcccagttttccataaatttatagataaaaagaatattttatattgcattttgtatgcatatatgcatacatacatatcacttaaatatatatatatataaaattgcatgttatgcacactttaaaatctttaaaatattgaatgcttaattacttaggacaaaatagcttacataggaaacaattatttcggacagaataatttaggagacaatagcatttttgtgctgttgcagagatgataaagaacttctggttttatatgtaactctaaaactgcaggataaataggtacgtaatacaaatggcagttgcctcactgcaattttctgagctgtgttgctagtctgacactcctgaaaattaatatttcagacatctctgtaattgtccagagggcctggagtgccttcaaattatattccccctctattttaatcaaccatgttagtaatttacttttcattagtttattgataattctatagggaaagtttgctaatcactgtgtaaaatataattttcaaacagccaaaataactgccataaaatatggaaactgtcttagtttgttttctcttgctatgaaagaataccacagactgggtaatgtatagagaagaggtttaaacactggccgtcgttttacaacgtcgtgactgggaaaaccctggcgttacccaacttaatcgccttgcagcacatccccctttcgccagctggcgtaatagcgaagaggcccgcaccgatcgcccttcccaacagttgcgcagcctgaatggcgaatggcgcctgatgcggtattttctccttacgcatctgtgcggtatttcacaccgcatatggtgcactctcagtacaatctgctctgatgccgcatagttaagccagccccgacacccgccaacacccgctgacgcgccctgacgggcttgtctgctcccggcatccgcttacagacaagctgtgaccgtctccgggagctgcatgtgtcagaggttttcaccgtcatcaccgaaacgcgcga

SEQ ID NO: 23 - DNA, 10761 bp, synthetic construct
  source 1..10761: mol_type = other DNA
tgcagctctggcccgtgtctcaaaatctctgatgttacattgcacaagataaaaatatatcatcatgaacaataaaactgtctgcttacataaacagtaatacaaggggtgttatgagccatattcaacgggaaacgtcgaggccgcgattaaattccaacatggatgctgatttatatgggtataaatgggctcgcgataatgtcgggcaatcaggtgcgacaatctatcgcttgtatgggaagcccgatgcgccagagttgtttctgaaacatggcaaaggtagcgttgccaatgatgttacagatgagatggtcagactaaactggctgacggaatttatgcctcttccgaccatcaagcattttatccgtactcctgatgatgcatggttactcaccactgcgatccccggaaaaacagcattccaggtattagaagaatatcctgattcaggtgaaaatattgttgatgcgctggcagtgttcctgcgccggttgcattcgattcctgtttgtaattgtccttttaacagcgatcgcgtatttcgtctcgctcaggcgcaatcacgaatgaataacggtttggttgatgcgagtgattttgatgacgagcgtaatggctggcctgttgaacaagtctggaaagaaatgcataaacttttgccattctcaccggattcagtcgtcactcatggtgatttctcacttgataaccttatttttgacgaggggaaattaataggttgtattgatgttggacgagtcggaatcgcagaccgataccaggatcttgccatcctatggaactgcctcggtgagttttctccttcattacagaaacggctttttcaaaaatatggtattgataatcctgatatgaataaattgcagtttcatttgatgctcgatgagtttttctaatcagaattggttaattggttgtaacattattcagattgggcttgatttaaaacttcatttttaatttaaaaggatctaggtgaagatcctttttgataatctcatgaccaaaatcccttaacgtgagttttcgttccactgagcgtcagaccccgtagaaaagatcaaaggatcttcttgagatcctttttttctgcgcgtaatctgctgcttgcaaacaaaaaaaccaccgctaccagcggtggtttgtttgccggatcaagagctaccaactctttttccgaaggtaactggcttcagcagagcgcagataccaaatactgttcttctagtgtagccgtagttaggccaccacttcaagaactctgtagcaccgcctacatacctcgctctgctaatcctgttaccagtggctgctgccagtggcgataagtcgtgtcttaccgggttggactcaagacgatagttaccggataaggcgcagcggtcgggctgaacggggggttcgtgcacacagcccagcttggagcgaacgacctacaccgaactgagatacctacagcgtgagctatgagaaagcgccacgcttcccgaagggagaaaggcggacaggtatccggtaagcggcagggtcggaacaggagagcgcacgagggagcttccagggggaaacgcctggtatctttatagtcctgtcgggtttcgccacctctgacttgagcgtcgatttttgtgatgctcgtcaggggggcggagcctatggaaaaacgccagcaacgcggcctttttacggttcctggccttttgctggccttttgctcacatgttctttcctgcgttatcccctgattctgtggataaccgtattaccgcctttgagtgagctgataccgctcgccgcagccgaacgaccgagcgcagcgagtcagtgagcgaggaagcggaagagcgcccaatacgcaaaccgcctctccccgcgcgttggccgattcattaatgcagctggcacgacaggtttcccgactggaaagcgggcagtgagcgcaacgcaattaatgtgagttagctcactcattaggcaccccaggctttacactttatgcttccggctcgtatgttgtgtggaattgtgagcggataacaatttcacacaggaaacagctatgaccatgattacgccgcggccgccagacacatgttccccagaagaggatttgccattctgacaaatctccatccaaggaatgggaaattcattatcccttccactagaattaaactgtgaaattatttatgtaggaagaagtagtagtagaaaagttatgtttgtcttcttcactataagaaaaaaatgcaaaatcaggaaaaatgtatctaaactattacttttacaaaggcaaaaacagcctgtttgctatctaatcagtcctgttgataaaactcaggctgtactgttctcttcagagagaggcaaatggggggagttataagatttgcgccctactgctgttagtagaatgaacaagacagagtaaaagccacaagtggaattgtgctagtatttcctctataattaacccaacacttaggtagcctttaaagtgaaaggagccctccaaatgatggaggcacacaggaggtaattatgtgctttcaataaatgcctgaaagctcacaatttctttggggagatacaatctctggaaaggcttgcattgtcactccaatttcatttatttattttaacaaattgtatgttctgtggaggaactttatttcccaaaaagatgaacgtataataaaccagttctttattttaaaacttatggtgagagaaatttcaattttagataattccattgtctataaagagtctctattaaattagcttaagttccaaaagataatgccacattattattgtaggtagccattataattctcaaatttctattgttacattctgcaagacagtggtaagcaaaccacaacggcggccgcataacttcgtatagcatacattatacgaagttatctgacctcttctcttcctcccacagggcctcgagagatctggcagcggagagggcagaggaagtcttctaacatgcggtgacgtggaggagaatcccggccctaggatgaccgagtacaagcccacggtgcgcctcgccacccgcgacgacgtccccagggccgtacgcaccctcgccgccgcgttcgccgactaccccgccacgcgccacaccgtcgatccggaccgccacatcgagcgggtcaccgagctgcaagaactcttcctcacgcgcgtcgggctcgacatcggcaaggtgtgggtcgcggacgacggcgccgcggtggcggtctggaccacgccggagagcgtcgaagcgggggcggtgttcgccgagatcggcccgcgcatggccgagttgagcggttcccggctggccgcgcagcaacagatggaaggcctcctggcgccgcaccggcccaaggagcccgcgtggttcctggccaccgtcggcgtctcgcccgaccaccagggcaagggtctgggcagcgccgtcgtgctccccggagtggaggcggccgagcgcgccggggtgcccgccttcctggagacctccgcgccccgcaacctccccttctacgagcggctcggcttcaccgtcaccgccgacgtcgaggtgcccgaaggaccgcgcacctggtgcatgacccgcaagcccggtgcctgactgtgccttctagttgccagccatctgttgtttgcccctcccccgtgccttccttgaccctggaaggtgccactcccactgtcctttcctaataaaatgaggaaattgcatcgcattgtctgagtaggtgtcattctattctggggggtggggtggggcaggacagcaagggggaggattgggaagacaatagcaggcatgctggggatgcggtgggctctatggataacttcgtatagcatacattatacgaagttatgagctcacggggacagcccccccccaaagcccccagggatgtaattacgtccctcccccgctagggggcagcagcgagccgcccggggctccgctccggtccggcgctccccccgcatccccgagccggcagcgtgcggggacagcccgggcacggggaaggtggcacgggatcgctttcctctgaacgcttctcgctgctctttgagcctgcagacacctggggggatacggggaaaaagctttaggctgaaagagagatttagaatgacagaatcatagaacggcctgggttgcaaaggagcacagtgctcatccagatccaaccccctgctatgtgcagggtcatcaaccagcagcccaggctgcccagagccacatccagcctggccttgaatgcctgcagggatggggcatccacagcctccttgggcaacctgttcagtgcgtcaccaccctctgggggaaaaactgcctcctcatatccaacccaaacctcccctgtctcagtgtaaagccattcccccttgtcctatcaagggggagtttgctgtgacattgttggtctggggtgacacatgtttgccaattcagtgcatcacggagaggcagatcttggggataaggaagtgcaggacagcatggacgtgggacatgcaggtgttgagggctctgggacactctccaagtcacagcgttcagaacagccttaaggataagaagataggatagaaggacaaagagcaagttaaaacccagcatggagaggagcacaaaaaggccacagacactgctggtccctgtgtctgagcctgcatgtttgatggtgtctggatgcaagcagaaggggtggaagagcttgcctggagagatacagctgggtcagtaggactgggacaggcagctggagaattgccatgtagatgttcatacaatcgtcaaatcatgaaggctggaaaagccctccaagatccccaagaccaaccccaacccacccaccgtgcccactggccatgtccctcagtgccacatccccacagttcttcatcacctccagggacggtgacccccccacctccgtgggcagctgtgccactgcagcaccgctctttggagaaggtaaatcttgctaaatccagcccgaccctcccctggcacaacgtaaggccattatctctcatccaactccaggacggagtcagtgagaatattggcgcgccgaattctcgcgacgatcggtcgacataacttcgtataggatactttatacgaagttatcaattcaggctagttattaatagtaatcaattacggggtcattagttcatagcccatatatggagttccgcgttacataacttacggtaaatggcccgcctggctgaccgcccaacgacccccgcccattgacgtcaataatgacgtatgttcccatagtaacgccaatagggactttccattgacgtcaatgggtggagtatttacggtaaactgcccacttggcagtacatcaagtgtatcatatgccaagtacgccccctattgacgtcaatgacggtaaatggcccgcctggcattatgcccagtacatgaccttatgggactttcctacttggcagtacatctacgtattagtcatcgctattaccatggtcgaggtgagccccacgttctgcttcactctccccatctcccccccctccccacccccaattttgtatttatttattttttaattattttgtgcagcgatgggggcggggggggggggggggcgcgcgccaggcggggcggggcggggcgaggggcggggcggggcgaggcggagaggtgcggcggcagccaatcagagcggcgcgctccgaaagtttccttttatggcgaggcggcggcggcggcggccctataaaaagcgaagcgcgcggcgggcggggagtcgctgcgacgctgccttcgccccgtgccccgctccgccgccgcctcgcgccgcccgccccggctctgactgaccgcgttactcccacaggtgagcgggcgggacggcccttctcctccgggctgtaattagcgcttggtttaatgacggcttgtttcttttctgtggctgcgtgaaagccttgaggggctccgggagggccctttgtgcggggggagcggctcggggggtgcgtgcgtgtgtgtgtgcgtggggagcgccgcgtgcggctccgcgctgcccggcggctgtgagcgctgcgggcgcggcgcggggctttgtgcgctccgcagtgtgcgcgaggggagcgcggccgggggcggtgccccgcggtgcggggggggctgcgaggggaacaaaggctgcgtgcggggtgtgtgcgtgggggggtgagcagggggtgtgggcgcgtcggtcgggctgcaaccccccctgcacccccctccccgagttgctgagcacggcccggcttcgggtgcggggctccgtacggggcgtggcgcggggctcgccgtgccgggcggggggtggcggcaggtgggggtgccgggcggggcggggccgcctcgggccggggagggctcgggggaggggcgcggcggcccccggagcgccggcggctgtcgaggcgcggcgagccgcagccattgccttttatggtaatcgtgcgagagggcgcagggacttcctttgtcccaaatctgtgcggagccgaaatctgggaggcgccgccgcaccccctctagcgggcgcggggcgaagcggtgcggcgccggcaggaaggaaatgggcggggagggccttcgtgcgtcgccgcgccgccgtccccttctccctctccagcctcggggctgtccgcggggggacggctgccttcgggggggacggggcagggcggggttcggcttctggcgtgtgaccggcggctctagagcctctgctaaccatgttcatgccttcttctttttcctacagctcctgggcaacgtgctggttattgtgctgtctcatcattttggcaaagaattgtgtacaaccatggagagcgacgagagcggcctgcccgccatggagatcgagtgccgcatcaccggcaccctgaacggcgtggagttcgagctggtgggcggcggagagggcacccccaagcagggccgcatgaccaacaagatgaagagcaccaaaggcgccctgaccttcagcccctacctgctgagccacgtgatgggctacggcttctaccacttcggcacctaccccagcggctacgagaaccccttcctgcacgccatcaacaacggcggctacaccaacacccgcatcgagaagtacgaggacggcggcgtgctgcacgtgagcttcagctaccgctacgaggccggccgcgtgatcggcgacttcaaggtggtgggcaccggcttccccgaggacagcgtgatcttcaccgacaagatcatccgcagcaacgccaccgtggagcacctgcaccccatgggcgataacgtgctggtgggcagcttcgcccgcaccttcagcctgcgcgacggcggctactacagcttcgtggtggacagccacatgcacttcaagagcgccatccaccccagcatcctgcagaacgggggccccatgttcgccttccgccgcgtggaggagctgcacagcaacaccgagctgggcatcgtggagtaccagcacgccttcaagacccccatcgccttcgccagatcccgcgctcagtcgtccaattctgccgtggacggcaccgccggacccggctccaccggatctcgctaaacgcgtgaattcactcctcaggtgcaggctgcctatcagaaggtggtggctggtgtggccaatgccctggctcacaaataccactgagatctttttccctctgccaaaaattatggggacatcatgaagccccttgagcatctgacttctggctaataaaggaaatttattttcattgcaatagtgtgttggaattttttgtgtctctcactcggaaggacatatgggagggcaaatcatttaaaacatcagaatgagtatttggtttagagtttggcaacatatgcccatatgctggctgccatgaacaaaggttggctataaagaggtcatcagtatatgaaacagccccctgctgtccattccttattccatagaaaagccttgacttgaggttagattttttttatattttgttttgtgttatttttttctttaacatccctaaaattttccttacatgttttactagccagatttttcctcctctcctgactactcccagtcatagctgtccctcttctcttatggagatcaccggtataacttcgtataatgtatactatacgaagttatggtaccttaattaagttaacatgcatagtactgagctcacggggacagcccccccccaaagcccccagggatgtaattacgtccctcccccgctagggggcagcagcgagccgcccggggctccgctccggtccggcgctccccccgcatccccgagccggcagcgtgcggggacagcccgggcacggggaaggtggcacgggatcgctttcctctgaacgcttctcgctgctctttgagcctgcagacacctggggggatacggggaaaaagctttaggctgaaagagagatttagaatgacagaatcatagaacggcctgggttgcaaaggagcacagtgctcatccagatccaaccccctgctatgtgcagggtcatcaaccagcagcccaggctgcccagagccacatccagcctggccttgaatgcctgcagggatggggcatccacagcctccttgggcaacctgttcagtgcgtcaccaccctctgggggaaaaactgcctcctcatatccaacccaaacctcccctgtctcagtgtaaagccattcccccttgtcctatcaagggggagtttgctgtgacattgttggtctggggtgacacatgtttgccaattcagtgcatcacggagaggcagatcttggggataaggaagtgcaggacagcatggacgtgggacatgcaggtgttgagggctctgggacactctccaagtcacagcgttcagaacagccttaaggataagaagataggatagaaggacaaagagcaagttaaaacccagcatggagaggagcacaaaaaggccacagacactgctggtccctgtgtctgagcctgcatgtttgatggtgtctggatgcaagcagaaggggtggaagagcttgcctggagagatacagctgggtcagtaggactgggacaggcagctggagaattgccatgtagatgttcatacaatcgtcaaatcatgaaggctggaaaagccctccaagatccccaagaccaaccccaacccacccaccgtgcccactggccatgtccctcagtgccacatccccacagttcttcatcacctccagggacggtgacccccccacctccgtgggcagctgtgccactgcagcaccgctctttggagaaggtaaatcttgctaaatccagcccgaccctcccctggcacaacgtaaggccattatctctcatccaactccaggacggagtcagtgagaatattgtttaaactctaggccaaatctggcctcccaattgttttataaataaaattttatttaaacgtaaccactcccattcatttgcttgtctctggttgtttttgcaatacaacagtagggttaggtagataatacaggctgtgtgtcacatgatgaagccaaaaacatttgctctctggctctttacagaatgaatttgcttatatttcttctaggatgtcaatttgtctgcttaattcacagaaggacaaattttaacataacttacttctatggcctgaatgtttgcgtacactgaaaattgatttgttgaaatcgatccccaatttgatagtattaggaggtagggctttggagatgtgattagatcatgagggtgtaacctttattaatgggattagtgcttttatatggggttgaagagacccgagctccccttccaccttgtgaggatgcagaaagaagatacattctgtgaactggaaagccggccctcactagacaccaaatatgccagtattttgatcttgggcttcccagccttcagaacttacagcagtccagaaagattaagacacccacctgaaatgttaattttgtcctaaaataatcttgcatttaagatctgaaatatgacctaagtattatctgaggagtcaatgctgatttattggtggtggatactgtgattctgtattaagaatggatctgaagccacataagataactgtgattacttagtgctattttcaatggctgtgagaagacaaccttgtgaccagaatttgaaaccctgcataaacaaaactcaacatgttttgaaggcctttacactcttcctctcagggtttaaacactggccgtcgttttacaacgtcgtgactgggaaaaccctggcgttacccaacttaatcgccttgcagcacatccccctttcgccagctggcgtaatagcgaagaggcccgcaccgatcgcccttcccaacagttgcgcagcctgaatggcgaatggcgcctgatgcggtattttctccttacgcatctgtgcggtatttcacaccgcatatggtgcactctcagtacaatctgctctgatgccgcatagttaagccagccccgacacccgccaacacccgctgacgcgccctgacgggcttgtctgctcccggcatccgcttacagacaagctgtgaccgtctccgggagctgcatgtgtcagaggttttcaccgtcatcaccgaaacgcgcga

SEQ ID NO: 24 - DNA, 10807 bp, synthetic construct
  source 1..10807: mol_type = other DNA
tgcagctctggcccgtgtctcaaaatctctgatgttacattgcacaagataaaaatatatcatcatgaacaataaaactgtctgcttacataaacagtaatacaaggggtgttatgagccatattcaacgggaaacgtcgaggccgcgattaaattccaacatggatgctgatttatatgggtataaatgggctcgcgataatgtcgggcaatcaggtgcgacaatctatcgcttgtatgggaagcccgatgcgccagagttgtttctgaaacatggcaaaggtagcgttgccaatgatgttacagatgagatggtcagactaaactggctgacggaatttatgcctcttccgaccatcaagcattttatccgtactcctgatgatgcatggttactcaccactgcgatccccggaaaaacagcattccaggtattagaagaatatcctgattcaggtgaaaatattgttgatgcgctggcagtgttcctgcgccggttgcattcgattcctgtttgtaattgtccttttaacagcgatcgcgtatttcgtctcgctcaggcgcaatcacgaatgaataacggtttggttgatgcgagtgattttgatgacgagcgtaatggctggcctgttgaacaagtctggaaagaaatgcataaacttttgccattctcaccggattcagtcgtcactcatggtgatttctcacttgataaccttatttttgacgaggggaaattaataggttgtattgatgttggacgagtcggaatcgcagaccgataccaggatcttgccatcctatggaactgcctcggtgagttttctccttcattacagaaacggctttttcaaaaatatggtattgataatcctgatatgaataaattgcagtttcatttgatgctcgatgagtttttctaatcagaattggttaattggttgtaacattattcagattgggcttgatttaaaacttcatttttaatttaaaaggatctaggtgaagatcctttttgataatctcatgaccaaaatcccttaacgtgagttttcgttccactgagcgtcagaccccgtagaaaagatcaaaggatcttcttgagatcctttttttctgcgcgtaatctgctgcttgcaaacaaaaaaaccaccgctaccagcggtggtttgtttgccggatcaagagctaccaactctttttccgaaggtaactggcttcagcagagcgcagataccaaatactgttcttctagtgtagccgtagttaggccaccacttcaagaactctgtagcaccgcctacatacctcgctctgctaatcctgttaccagtggctgctgccagtggcgataagtcgtgtcttaccgggttggactcaagacgatagttaccggataaggcgcagcggtcgggctgaacggggggttcgtgcacacagcccagcttggagcgaacgacctacaccgaactgagatacctacagcgtgagctatgagaaagcgccacgcttcccgaagggagaaaggcggacaggtatccggtaagcggcagggtcggaacaggagagcgcacgagggagcttccagggggaaacgcctggtatctttatagtcctgtcgggtttcgccacctctgacttgagcgtcgatttttgtgatgctcgtcaggggggcggagcctatggaaaaacgccagcaacgcggcctttttacggttcctggccttttgctggccttttgctcacatgttctttcctgcgttatcccctgattctgtggataaccgtattaccgcctttgagtgagctgataccgctcgccgcagccgaacgaccgagcgcagcgagtcagtgagcgaggaagcggaagagcgcccaatacgcaaaccgcctctccccgcgcgttggccgattcattaatgcagctggcacgacaggtttcccgactggaaagcgggcagtgagcgcaacgcaattaatgtgagttagctcactcattaggcaccccaggctttacactttatgcttccggctcgtatgttgtgtggaattgtgagcggataacaatttcacacaggaaacagctatgaccatgattacgccgcggccgcggcttccctctgtgatgggtagataattttgcttaatatgtaaacagtcttttcaacactctgtgcttaaataatcattgttggtttgctttcttctagtattccatattaagtaatgacttggctaatgagaaggatgcttgtaagtatattagcatcaagttcaaatatagagagattaaataaccttcccaaggtcaacacactggtcattgacaaatatggaccagatctcatctccaaaaccccacacaattataccaggttagctcattctttcttcctagacatcttattttccagggagtagtgaaggtctacaaaactttcctactaaataggaaatatattttgttgtcagatgtaagcccagaaaagcaatggctaaactgctatgtatcaaaaactttgcaaacttataacagtttaaaatttacttctagctatgtttagagccctaaggagataatggcaagtcattttttcttctttatacatatgtcatcatttatggacagaaaatagttctcaattgtaaaaaaatagctctctataggatttgctgagttttttatggctagagttattaagtaaaataaatgacatctgagagcactctgctttgtctttggcttcaaataatgtattttactatattttttcattcttcgctgccataagtggcagaaagaaaaccgcttttcaaatggctagtgcctaaaaagcaaatactttgtggatcttggggccagtgtaaactcagaatgcaagatatcttcctcagcttcagtacttgcacaatgcctgtctttattaaacatgagtgatttgcaaatatgatgtttctgagacagctaatagcggccgcataacttcgtatagcatacattatacgaagttatctgacctcttctcttcctcccacagggcctcgagagatctggcagcggagagggcagaggaagtcttctaacatgcggtgacgtggaggagaatcccggccctaggatgaccgagtacaagcccacggtgcgcctcgccacccgcgacgacgtccccagggccgtacgcaccctcgccgccgcgttcgccgactaccccgccacgcgccacaccgtcgatccggaccgccacatcgagcgggtcaccgagctgcaagaactcttcctcacgcgcgtcgggctcgacatcggcaaggtgtgggtcgcggacgacggcgccgcggtggcggtctggaccacgccggagagcgtcgaagcgggggcggtgttcgccgagatcggcccgcgcatggccgagttgagcggttcccggctggccgcgcagcaacagatggaaggcctcctggcgccgcaccggcccaaggagcccgcgtggttcctggccaccgtcggcgtctcgcccgaccaccagggcaagggtctgggcagcgccgtcgtgctccccggagtggaggcggccgagcgcgccggggtgcccgccttcctggagacctccgcgccccgcaacctccccttctacgagcggctcggcttcaccgtcaccgccgacgtcgaggtgcccgaaggaccgcgcacctggtgcatgacccgcaagcccggtgcctgactgtgccttctagttgccagccatctgttgtttgcccctcccccgtgccttccttgaccctggaaggtgccactcccactgtcctttcctaataaaatgaggaaattgcatcgcattgtctgagtaggtgtcattctattctggggggtggggtggggcaggacagcaagggggaggattgggaagacaatagcaggcatgctggggatgcggtgggctctatggataacttcgtatagcatacattatacgaagttatgagctcacggggacagcccccccccaaagcccccagggatgtaattacgtccctcccccgctagggggcagcagcgagccgcccggggctccgctccggtccggcgctccccccgcatccccgagccggcagcgtgcggggacagcccgggcacggggaaggtggcacgggatcgctttcctctgaacgcttctcgctgctctttgagcctgcagacacctggggggatacggggaaaaagctttaggctgaaagagagatttagaatgacagaatcatagaacggcctgggttgcaaaggagcacagtgctcatccagatccaaccccctgctatgtgcagggtcatcaaccagcagcccaggctgcccagagccacatccagcctggccttgaatgcctgcagggatggggcatccacagcctccttgggcaacctgttcagtgcgtcaccaccctctgggggaaaaactgcctcctcatatccaacccaaacctcccctgtctcagtgtaaagccattcccccttgtcctatcaagggggagtttgctgtgacattgttggtctggggtgacacatgtttgccaattcagtgcatcacggagaggcagatcttggggataaggaagtgcaggacagcatggacgtgggacatgcaggtgttgagggctctgggacactctccaagtcacagcgttcagaacagccttaaggataagaagataggatagaaggacaaagagcaagttaaaacccagcatggagaggagcacaaaaaggccacagacactgctggtccctgtgtctgagcctgcatgtttgatggtgtctggatgcaagcagaaggggtggaagagcttgcctggagagatacagctgggtcagtaggactgggacaggcagctggagaattgccatgtagatgttcatacaatcgtcaaatcatgaaggctggaaaagccctccaagatccccaagaccaaccccaacccacccaccgtgcccactggccatgtccctcagtgccacatccccacagttcttcatcacctccagggacggtgacccccccacctccgtgggcagctgtgccactgcagcaccgctctttggagaaggtaaatcttgctaaatccagcccgaccctcccctggcacaacgtaaggccattatctctcatccaactccaggacggagtcagtgagaatattggcgcgccgaattctcgcgacgatcggtcgacataacttcgtataggatactttatacgaagttatcaattcaggctagttattaatagtaatcaattacggggtcattagttcatagcccatatatggagttccgcgttacataacttacggtaaatggcccgcctggctgaccgcccaacgacccccgcccattgacgtcaataatgacgtatgttcccatagtaacgccaatagggactttccattgacgtcaatgggtggagtatttacggtaaactgcccacttggcagtacatcaagtgtatcatatgccaagtacgccccctattgacgtcaatgacggtaaatggcccgcctggcattatgcccagtacatgaccttatgggactttcctacttggcagtacatctacgtattagtcatcgctattaccatggtcgaggtgagccccacgttctgcttcactctccccatctcccccccctccccacccccaattttgtatttatttattttttaattattttgtgcagcgatgggggcggggggggggggggggcgcgcgccaggcggggcggggcggggcgaggggcggggcggggcgaggcggagaggtgcggcggcagccaatcagagcggcgcgctccgaaagtttccttttatggcgaggcggcggcggcggcggccctataaaaagcgaagcgcgcggcgggcggggagtcgctgcgacgctgccttcgccccgtgccccgctccgccgccgcctcgcgccgcccgccccggctctgactgaccgcgttactcccacaggtgagcgggcgggacggcccttctcctccgggctgtaattagcgcttggtttaatgacggcttgtttcttttctgtggctgcgtgaaagccttgaggggctccgggagggccctttgtgcggggggagcggctcggggggtgcgtgcgtgtgtgtgtgcgtggggagcgccgcgtgcggctccgcgctgcccggcggctgtgagcgctgcgggcgcggcgcggggctttgtgcgctccgcagtgtgcgcgaggggagcgcggccgggggcggtgccccgcggtgcggggggggctgcgaggggaacaaaggctgcgtgcggggtgtgtgcgtgggggggtgagcagggggtgtgggcgcgtcggtcgggctgcaaccccccctgcacccccctccccgagttgctgagcacggcccggcttcgggtgcggggctccgtacggggcgtggcgcggggctcgccgtgccgggcggggggtggcggcaggtgggggtgccgggcggggcggggccgcctcgggccggggagggctcgggggaggggcgcggcggcccccggagcgccggcggctgtcgaggcgcggcgagccgcagccattgccttttatggtaatcgtgcgagagggcgcagggacttcctttgtcccaaatctgtgcggagccgaaatctgggaggcgccgccgcaccccctctagcgggcgcggggcgaagcggtgcggcgccggcaggaaggaaatgggcggggagggccttcgtgcgtcgccgcgccgccgtccccttctccctctccagcctcggggctgtccgcggggggacggctgccttcgggggggacggggcagggcggggttcggcttctggcgtgtgaccggcggctctagagcctctgctaaccatgttcatgccttcttctttttcctacagctcctgggcaacgtgctggttattgtgctgtctcatcattttggcaaagaattgtgtacaaccatggagagcgacgagagcggcctgcccgccatggagatcgagtgccgcatcaccggcaccctgaacggcgtggagttcgagctggtgggcggcggagagggcacccccaagcagggccgcatgaccaacaagatgaagagcaccaaaggcgccctgaccttcagcccctacctgctgagccacgtgatgggctacggcttctaccacttcggcacctaccccagcggctacgagaaccccttcctgcacgccatcaacaacggcggctacaccaacacccgcatcgagaagtacgaggacggcggcgtgctgcacgtgagcttcagctaccgctacgaggccggccgcgtgatcggcgacttcaaggtggtgggcaccggcttccccgaggacagcgtgatcttcaccgacaagatcatccgcagcaacgccaccgtggagcacctgcaccccatgggcgataacgtgctggtgggcagcttcgcccgcaccttcagcctgcgcgacggcggctactacagcttcgtggtggacagccacatgcacttcaagagcgccatccaccccagcatcctgcagaacgggggccccatgttcgccttccgccgcgtggaggagctgcacagcaacaccgagctgggcatcgtggagtaccagcacgccttcaagacccccatcgccttcgccagatcccgcgctcagtcgtccaattctgccgtggacggcaccgccggacccggctccaccggatctcgctaaacgcgtgaattcactcctcaggtgcaggctgcctatcagaaggtggtggctggtgtggccaatgccctggctcacaaataccactgagatctttttccctctgccaaaaattatggggacatcatgaagccccttgagcatctgacttctggctaataaaggaaatttattttcattgcaatagtgtgttggaattttttgtgtctctcactcggaaggacatatgggagggcaaatcatttaaaacatcagaatgagtatttggtttagagtttggcaacatatgcccatatgctggctgccatgaacaaaggttggctataaagaggtcatcagtatatgaaacagccccctgctgtccattccttattccatagaaaagccttgacttgaggttagattttttttatattttgttttgtgttatttttttctttaacatccctaaaattttccttacatgttttactagccagatttttcctcctctcctgactactcccagtcatagctgtccctcttctcttatggagatcaccggtataacttcgtataatgtatactatacgaagttatggtaccttaattaagttaacatgcatagtactgagctcacggggacagcccccccccaaagcccccagggatgtaattacgtccctcccccgctagggggcagcagcgagccgcccggggctccgctccggtccggcgctccccccgcatccccgagccggcagcgtgcggggacagcccgggcacggggaaggtggcacgggatcgctttcctctgaacgcttctcgctgctctttgagcctgcagacacctggggggatacggggaaaaagctttaggctgaaagagagatttagaatgacagaatcatagaacggcctgggttgcaaaggagcacagtgctcatccagatccaaccccctgctatgtgcagggtcatcaaccagcagcccaggctgcccagagccacatccagcctggccttgaatgcctgcagggatggggcatccacagcctccttgggcaacctgttcagtgcgtcaccaccctctgggggaaaaactgcctcctcatatccaacccaaacctcccctgtctcagtgtaaagccattcccccttgtcctatcaagggggagtttgctgtgacattgttggtctggggtgacacatgtttgccaattcagtgcatcacggagaggcagatcttggggataaggaagtgcaggacagcatggacgtgggacatgcaggtgttgagggctctgggacactctccaagtcacagcgttcagaacagccttaaggataagaagataggatagaaggacaaagagcaagttaaaacccagcatggagaggagcacaaaaaggccacagacactgctggtccctgtgtctgagcctgcatgtttgatggtgtctggatgcaagcagaaggggtggaagagcttgcctggagagatacagctgggtcagtaggactgggacaggcagctggagaattgccatgtagatgttcatacaatcgtcaaatcatgaaggctggaaaagccctccaagatccccaagaccaaccccaacccacccaccgtgcccactggccatgtccctcagtgccacatccccacagttcttcatcacctccagggacggtgacccccccacctccgtgggcagctgtgccactgcagcaccgctctttggagaaggtaaatcttgctaaatccagcccgaccctcccctggcacaacgtaaggccattatctctcatccaactccaggacggagtcagtgagaatattgtttaaactcatgggccaaaatgaatggaatcaaaacctgagacacatttctgttaatggggctctatttgagaaatgtgcattattttatcagcttccttattttaaccattctaccctgtcaatactaataccaagtgttcattttctttattagtttaaatgggagaaaacaatgcagaaagcttaataactgttctatttttaaagcctttatagaaaacataatataaaaagtgatatgaactaggcacaagacaaaactgactttaatatgttatatgttaatctgttaaaatacagtacattttactgcagaatgttagcagggtatatttgtagataatagatcattgacatttttatcctatatcctttttaccttttattccttttaaacattgattacctttgttataaaaagcaacaacaatagtttgtaaaagattaagatatttaaatatttaaaaatttttcataactatattagtaaacagtagtacataagtcttgataggtacaaatgatgtctcaaaagacagatgaggtggaaaattaccactctagctcatggcatgaccccagccgtgcagaggaaagatttcttctcctcccctattcacctccgggtcccagctatcactaaatatatcgggggtcgcgttgctgatcagcagccttaagcctgaacatggtgggtcctttgcattagttctcaattcccaccaccctcctcccttcctgtgtcacgaggctcactcatttcctcagtgcccttcccagttactgtcaaatcatataaactcatttctctgcctccagccttttatttcatcgtttaaacactggccgtcgttttacaacgtcgtgactgggaaaaccctggcgttacccaacttaatcgccttgcagcacatccccctttcgccagctggcgtaatagcgaagaggcccgcaccgatcgcccttcccaacagttgcgcagcctgaatggcgaatggcgcctgatgcggtattttctccttacgcatctgtgcggtatttcacaccgcatatggtgcactctcagtacaatctgctctgatgccgcatagttaagccagccccgacacccgccaacacccgctgacgcgccctgacgggcttgtctgctcccggcatccgcttacagacaagctgtgaccgtctccgggagctgcatgtgtcagaggttttcaccgtcatcaccgaaacgcgcga

SEQ ID NO: 25 - DNA, 10760 bp, synthetic construct; identical to SEQ ID NO: 2
  source 1..10760: mol_type = other DNA